European Patent Application EP 4 321 618 A1, published February 14, 2024. Title: VARIANTS OF TEV PROTEASE AND USES THEREOF. Applicant: Numaferm GmbH. The sequence listing filed with the application follows.

SEQUENCE LISTING (23 sequences)

SEQ ID NO: 1 - protein, 236 aa, synthetic construct
  REGION 1..236: note = TEV protease mutant
GESLFKGPRDYNPISSSICHLTNESDGHTTSLYGIGFGPFIITNKHLFRRNNGTLLVQSLHGVFKVKDTTTLQQHLVDGRDMIIIRMPKDFPPFPQKLKFREPQREERICLVTTNFQTKSMSSMVSDTSCTFPSSDGIFWKHWIQTKDGQCGSPLVSTRDGFIVGIHSASNFTNTNNYFTSVPKNFMELLTNQEAQQWVSGWRLNADSVLWGGHKVFMNKPEEPFQPVKEATQLMN

SEQ ID NO: 2 - protein, 242 aa, Tobacco etch virus
GESLFKGPRDYNPISSTICHLTNESDGHTTSLYGIGFGPFIITNKHLFRRNNGTLLVQSLHGVFKVKNTTTLQQHLIDGRDMIIIRMPKDFPPFPQKLKFREPQREERICLVTTNFQTKSMSSMVSDTSCTFPSSDGIFWKHWIQTKDGQCGSPLVSTRDGFIVGIHSASNFTNTNNYFTSVPKNFMELLTNQEAQQWVSGWRLNADSVLWGGHKVFMSKPEEPFQPVKEATQLMNELVYSQ

SEQ ID NO: 3 - protein, 236 aa, synthetic construct
  REGION 1..236: note = TEV protease DM
GESLFKGPRDYNPISSSICHLTNESDGHTTSLYGIGFGPFIITNKHLFRRNNGTLLVQSLHGVFKVKDTTTLQQHLVDGRDMIIIRMPKDFPPFPQKLKFREPQREERICLVTTNFQTKSMSSMVSDTSCTFPSSDGIFWKHWIQTKDGQCGNPLVSTRDGFIVGIHSASNFTNTNNYFTSVPKNFMELLTNQEAQQWVSGWGLNADSVLWGGHKVFMNKPEEPFQPVKEATQLMN

SEQ ID NO: 4 - protein, 236 aa, synthetic construct
  REGION 1..236: note = TEV mutant clone 1
GESLFKGPRDYNPISSSICHLVNESDGHTASLYGIGFGPFIITNKHLFRRNNGTLLVQSLHGVFKVKDTTTLQQHLVDGRDMIIIRMPKDFPPFPQKLKFREPQREERICLVTTNFQTKSMSSMVSDTSCTFPSSDGIFWKHWIQTKNGQCGSPLVSTRDGFIVGIHSASNFTNTNNYFTSVPKNFMELLTNQEAQQWVSGWGLNADSVLWGGHKVFFNKPEEPFQPVKEATQLMN

SEQ ID NO: 5 - protein, 236 aa, synthetic construct
  REGION 1..236: note = TEV mutant clone 4
GESLFKGPRDYNPISSSICHLSNESDGHTASLYGIGFGPFIITNKHLFRRNNGTLLVQSLHGVFKVKDTTTLQQHLVDGRDMIIIRMPKDFPPFPQKLKFREPQREERICLVTTNFQTKSMSSMVSDTSCTFPSSDGIFWKHWIQTKNGQCGSPLVSTRDGFIVGIHSASNFTNTNNYFTSVPKNFMELLTNQEAQQWVSGWGLNADSVLWGGHKVFFNKPEEPFQPVKEATQLMN

SEQ ID NO: 6 - protein, 236 aa, synthetic construct
  REGION 1..236: note = TEV mutant clone 2
GESLFKGPRDYNPISSSICHLINESDGHTASLYGIGFGPFIITNKHLFRRNNGTLLVQSLHGVFKVKDTTTLQQHLVDGRDMIIIRMPKDFPPFPQKLKFREPQREERICLVTTNFQTKSMSSMVSDTSCTFPSSDGIFWKHWIQTKDGQCGSPLVSTRDGFIVGIHSASNFTNTNNYFTSVPKNFMELLTNQEAQQWVSGWGLNADSVLWGGHKVFFNKPEEPFQPVKEATQLMN

SEQ ID NO: 7 - protein, 236 aa, synthetic construct
  REGION 1..236: note = TEV mutant clone 8
GESLFKGPRDYNPISSSICHLINESDGHTASLYGIGFGPFIITNKHLFRRNNGTLLVQSLHGVFKVKDTTTLQQHLVDGRDMIIIRMPKDFPPFPQKLKFREPQREERICLVTTNFQTKSMSSMVSDTSCTFPSSDGIFWKHWIQTKRGQCGSPLVSTRDGFIVGIHSASNFTNTNNYFTSVPKNFMELLTNQEAQQWVSGWGLNADSVLWGGHKVFFNKPEEPFQPVKEATQLMN

SEQ ID NO: 8 - protein, 236 aa, synthetic construct
  REGION 1..236: note = TEV mutant clone 11
GESLFKGPRDYNPISSSICHLYNESDGHTSSLYGIGFGPFIITNKHLFRRNNGTLLVQSLHGVFKVKDTTTLQQHLVDGRDMIIIRMPKDFPPFPQKLKFREPQREERICLVTTNFQTKSMSSMVSDTSCTFPSSDGIFWKHWIQTKNGQCGSPLVSTRDGFIVGIHSASNFTNTNNYFTSVPKNFMELLTNQEAQQWVSGWGLNADSVLWGGHKVFFNKPEEPFQPVKEATQLMN

SEQ ID NO: 9 - protein, 236 aa, synthetic construct
  REGION 1..236: note = TEV mutant clone 19
GESLFKGPRDYNPISSSICHLINESDGHTSSLYGIGFGPFIITNKHLFRRNNGTLLVQSLHGVFKVKDTTTLQQHLVDGRDMIIIRMPKDFPPFPQKLKFREPQREERICLVTTNFQTKSMSSMVSDTSCTFPSSDGIFWKHWIQTKYGQCGSPLVSTRDGFIVGIHSASNFTNTNNYFTSVPKNFMELLTNQEAQQWVSGWGLNADSVLWGGHKVFFNKPEEPFQPVKEATQLMN

SEQ ID NO: 10 - protein, 236 aa, synthetic construct
  REGION 1..236: note = TEV mutant clone 20
GESLFKGPRDYNPISSSICHLYNESDGHTSSLYGIGFGPFIITNKHLFRRNNGTLLVQSLHGVFKVKDTTTLQQHLVDGRDMIIIRMPKDFPPFPQKLKFREPQREERICLVTTNFQTKSMSSMVSDTSCTFPSSDGIFWKHWIQTKRGQCGSPLVSTRDGFIVGIHSASNFTNTNNYFTSVPKNFMELLTNQEAQQWVSGWGLNADSVLWGGHKVFFNKPEEPFQPVKEATQLMN

SEQ ID NO: 11 - protein, 236 aa, synthetic construct
  REGION 1..236: note = TEV mutant clone 16
GESLFKGPRDYNPISSSICHLINESDGHTSSLYGIGFGPFIITNKHLFRRNNGTLLVQSLHGVFKVKDTTTLQQHLVDGRDMIIIRMPKDFPPFPQKLKFREPQREERICLVTTNFQTKSMSSMVSDTSCTFPSSDGIFWKHWIQTKDGQCGSPLVSTRDGFIVGIHSASNFTNTNNYFTSVPKNFMELLTNQEAQQWVSGWGLNADSVLWGGHKVFFNKPEEPFQPVKEATQLMN

SEQ ID NO: 12 - protein, 236 aa, synthetic construct
  REGION 1..236: note = TEV mutant clone 17
GESLFKGPRDYNPISSSICHLINESDGHTSSLYGIGFGPFIITNKHLFRRNNGTLLVQSLHGVFKVKDTTTLQQHLVDGRDMIIIRMPKDFPPFPQKLKFREPQREERICLVTTNFQTKSMSSMVSDTSCTFPSSDGIFWKHWIQTKRGQCGSPLVSTRDGFIVGIHSASNFTNTNNYFTSVPKNFMELLTNQEAQQWVSGWGLNADSVLWGGHKVFFNKPEEPFQPVKEATQLMN

SEQ ID NO: 13 - protein, 236 aa, synthetic construct
  REGION 1..236: note = TEV mutant clone P1
GESLFKGPRDYNPISSSICHLTNESDGHTTSLYGIGFGPFIITNKHLFRRNNGTLLVQSLHGVFKVKDTTTLQLHLVDGRDMIIIRMPKDFPPFPQKLKFREPQREERICLVTTNFQTKSMSSMVSDTSCTFPSGDGTFWKHWIQTKDGQCGNPLVSTRDGFIVGIHSASNFTNTNNYFTSVPKNFMELLTNQEAQQWVSGWGLNADSVLWGGHKVFMNKPEEPFQPVKEATQLMN

SEQ ID NO: 14 - protein, 236 aa, synthetic construct
  REGION 1..236: note = TEV mutant clone P3
GESLCKGPRDYNPISSSICHLTNESDGHTTSLYGIGFGPFIITNKHLFRRNNGTLLVQSWHGVFKVKDTTTLQLHLVDGRDMIIIRMPKDFPPFPQKLKFREPQREERICLVTTNFQTKSMSSMVSDTSCTFPSGDGHFWKHWIQTKDGQCGNPLVSTRDGFIVGIHSASNFTNTNNYFTSVPKNFMELLTNQEAQQWVSGWGLNADSVCWGGHKVFMNKPEEPFQPVKEATQLMN

SEQ ID NO: 15 - protein, 236 aa, synthetic construct
  REGION 1..236: note = TEV mutant clone P4
GESLCKGPRDYNPISSSICHLTNESDGHTTSLYGIGFGPFIITNKHLFRRNNGTLLVQSWHGVFKVKDTTTLQLHPVDGRDMIIIRMPKDFPPFPQKLKFREPQREERICLVTTNFQTKSMSSMVSDTSTTFPSGDGHFWKHWIQTKDGQCGNPLVSTRDGFIVGIHSASNFTNTNNYFTSVPKNFMELLTNQEAQQWVKGWGLNTDSVCWGGHKVFMNKPEEPFQPVKEATQLMN

SEQ ID NO: 16 - protein, 236 aa, synthetic construct
  REGION 1..236: note = TEV mutant clone P5
GESLCKGPRDYNPISSSICHLTNESDGHTTSLYGIGFGPFIITNKHLFRRNNGTLLVQSWHGVFKVKDTTTLQLHPVEGRDMIIIRMPKDFPPFPQKLKFREPQREERICLVGTNFQEKSMSSMVSETSTTFPSGDGHFWKHWIQTKDGQCGNPLVSTRDGFIVGIHSASNFTNTNNYFTSVPKNFMELLTNQEAQQWVKGWGLNTDSVCWGGHKVFMNKPEEPFQPVKEATQLMN

SEQ ID NO: 17 - protein, 236 aa, synthetic construct
  REGION 1..236: note = TEV mutant clone P1rev
GESLFKGPRDYNPISSSICHLTNESDGHTTSLYGIGFGPFIITNKHLFRRNNGTLLVQSLHGVFKVKDTTTLQLHLVDGRDMIIIRMPKDFPPFPQKLKFREPQREERICLVTTNFQTKSMSSMVSDTSCTFPSGDGTFWKHWIQTKDGQCGSPLVSTRDGFIVGIHSASNFTNTNNYFTSVPKNFMELLTNQEAQQWVSGWGLNADSVLWGGHKVFMNKPEEPFQPVKEATQLMN

SEQ ID NO: 18 - protein, 7 aa, synthetic construct
  REGION 1..7: note = TEV recognition site
  SITE 7: note = misc_feature - Xaa can be any naturally occurring amino acid
ENLYFQX

SEQ ID NO: 19 - protein, 10 aa, synthetic construct
  REGION 1..10: note = Gly peptide substrate
ENLYFQGGGK

SEQ ID NO: 20 - protein, 10 aa, synthetic construct
  REGION 1..10: note = Val peptide substrate
ENLYFQVGGK

SEQ ID NO: 21 - protein, 14 aa, synthetic construct
  REGION 1..14: note = N terminal tag
GTHHHHHHGSGSGT

SEQ ID NO: 22 - protein, 10 aa, synthetic construct
  REGION 1..10: note = TEV substrate peptide
  SITE 7: note = misc_feature - Xaa can be any naturally occurring amino acid
ENLYFQXGGK

SEQ ID NO: 23 - protein, 250 aa, synthetic construct
GTHHHHHHGSGSGTGESLHKGPRDYNNIASSICLLTNESDGHTTSLYGIGFGPYIITNKHLFRRNNGTLKVQSHHGVFKVPDTTTLQLHFVEGRDMIIIRMPKDFPPFPQKLKFREPQRNERICLVGTNFQEKSLSTMVSETSTTYPVGDGTFWKHWIQTKDGQCGNPMVSTKDGAIVGIHSASNFTNTNNYFTSIPKNFMELLTNPEAQDWVKGWGYNADSVLWGGHKVFMNKPEEPFQPVKEATQLMN